European Patent Specification EP 3 886 881 B1, published July 16, 2025. Title: BACTERIAL STRAINS FOR MEDICAL USES. Applicant: Ospedale San Raffaele S.r.l. The sequence listing filed with the application follows.

SEQUENCE LISTING (2 sequences)

SEQ ID NO: 1 - DNA, 23 bp, Artificial Sequence
  synthetic
acagctacggaactcttgtgcgt

SEQ ID NO: 2 - DNA, 23 bp, Artificial Sequence
  synthetic
tcagccaaggttgtgaggttgca